European Patent Application EP 4 265 277 A1, published October 25, 2023. Title: Composition for Preventing or Treating Glioblastoma Comprising Peptide Nucleic Acid Complex. Applicant: SEASUN THERAPEUTICS, INC. The sequence listing filed with the application follows.

SEQUENCE LISTING (10 sequences)

SEQ ID NO: 1 - DNA, 15 bp, Artificial Sequence
  bioactive 1
aactggtccatatcg

SEQ ID NO: 2 - DNA, 15 bp, Artificial Sequence
  bioactive 2
  misc_feature (1): GLFDIIKKIAESF
aactggtccatatcg

SEQ ID NO: 3 - DNA, 15 bp, Artificial Sequence
  bioactive 3
tatatcggtctaagc

SEQ ID NO: 4 - DNA, 15 bp, Artificial Sequence
  carrier 1
ttgaccaggtatagc

SEQ ID NO: 5 - DNA, 15 bp, Artificial Sequence
  carrier 2
cgatatggaccagtt

SEQ ID NO: 6 - DNA, 5 bp, Artificial Sequence
  carrier 3
atagc

SEQ ID NO: 7 - DNA, 5 bp, Artificial Sequence
  carrier 4
cgata

SEQ ID NO: 8 - DNA, 15 bp, Artificial Sequence
  carrier 5
atatagccagattcg

SEQ ID NO: 9 - DNA, 15 bp, Artificial Sequence
  carrier 6
cgatatggaccagtt

SEQ ID NO: 10 - protein, 13 aa, Artificial Sequence
  endosome escaper
GLFDIIKKIAESF